European Patent Application EP 4 796 559 A1, published August 26, 2026. Title: 一种角蛋白CF6、制法和其药物组合物与用途. Applicant: 中国医学科学院药物研究所. The sequence listing filed with the application follows.

SEQUENCE LISTING (2 sequences)

SEQ ID NO: 1 - protein, 529 aa, unidentified
MTCGFSSVGCGFSPRTFSCASACGPRPGRCCITAAPYRGVSCYRGLCGGFGSRSLCGGFRAGSCGRSFGYRSGGVRGPSAPCITTVSVNESLLAPLNLEIDPNAQYVKQEEKEQIKSLNNRFAAFIDKVRFLEQQNKLLETKLQFYQNRKCCDSNLEPLFSGYLEALWREAECVEADSGRLASELSHVQEVLEGYKKRYEEEVTLRATAENEFVALKKDVDCAYLRKSDLEANAEALTQEVDFLRRLYEEEIRVLQAHISDTSVIVKMDNSRDLNLASIVAEIKAHYDDIASRSRAEAESWYRTKCEEIKATVVRHGETLRRTKEEINELNRLIQQLTAEIENAKCQNSKLEAAVAEAEQQGEAALNDARCKLAGLEDALQKAKQDMACLLREYQEVLNSKLGLDIEIATYRRLLEGEEQRAGAGEGEGGGAEGLPSSWAQQPRILKQNSSTCHSQQPLSACGRQETRRGIPVQGERRSGQQGRWVRVRSSSCTHHQAAHGRVGQKGRLGSSGSVRGLGAWVLPQALPA

SEQ ID NO: 2 - DNA, 1587 bp, unidentified
  source 1..1587: mol_type = other DNA
atgacctgcggctttagcagcgttggctgcggctttagcccgcgtacctttagctgtgcgagcgcgtgtggtcctcgcccaggtcgttgttgtattaccgcggcgccttatcgcggtgttagctgttatcgtggcctgtgtggcggctttggtagccgcagcctgtgtggtggttttcgtgcgggttcatgtggtcgtagctttggctatcgcagcggcggcgttcgtggtccttcagcgccttgtattaccaccgttagcgttaacgaaagcctgctggcgccgttaaacctggaaattgatccgaacgcgcagtatgtgaaacaggaagaaaaagaacagatcaagagcctgaacaaccgctttgcggcgtttattgataaagtgcgctttctggaacagcagaacaaactgctggaaaccaaactgcagttttatcagaaccgcaaatgctgcgatagcaacctggaaccgctgtttagcggctatctggaagcgctgtggcgcgaagcagaatgcgttgaagcggatagcggccgtttagcgagcgaattaagccatgtgcaggaagtgctggaaggctataaaaaacgctatgaagaagaggtgaccctgcgcgcgaccgcggaaaatgaatttgtggcgctgaaaaaagatgtggactgcgcgtatctgcgcaaaagcgatctggaagcgaacgcggaagcgctgacccaagaagttgattttctgcgccgcctgtatgaagaagaaattcgcgtgctgcaggcgcatattagcgataccagcgtgattgtgaaaatggataacagccgcgatctgaacctggcgagcattgtggcggaaattaaagcgcattatgatgacattgcgagccgcagccgcgcggaagcggaaagctggtatcgtactaaatgcgaagaaattaaggcgaccgtggtgcgccatggcgaaaccttacgtcgcaccaaagaagaaattaacgaactgaaccgcctgattcagcagctgaccgcggaaattgaaaacgcgaaatgccagaacagcaaactggaagcggcggtggcggaagcggaacaacaaggcgaagcggcgttaaacgatgcgcgctgtaaactggcgggcttagaagatgcgctgcagaaagcgaaacaggatatggcgtgcctgctgcgcgaatatcaggaagtgctgaacagcaaactgggcctggatattgaaattgcgacctatcgccgcctgctggaaggcgaagaacagcgcgcgggtgcgggtgaaggtgaaggtggtggtgcggaaggtttaccttcaagctgggcgcagcaacctcgtattttaaaacagaacagcagcacctgccatagccagcagccgttaagcgcgtgtggccgtcaagaaacccgtcgcggtattccggttcagggtgaacgccgtagcggccaacaaggccgttgggttcgtgttcgcagcagctcatgtacccatcatcaggcggcgcatggtcgcgttggtcaaaaaggtcgtttaggcagcagcggtagcgtgcgtggtctgggtgcatgggtgttaccgcaagcgttacctgcg